European Patent Specification EP 3 642 362 B1, published October 15, 2025. Title: METHODS AND COMPOSITIONS FOR ADDRESSING INEFFICIENCIES IN AMPLIFICATION REACTIONS. Applicant: ILLUMINA, INC. The sequence listing filed with the application follows.

SEQUENCE LISTING (468 sequences)

SEQ ID NO: 1 - DNA, 19 bp, Artificial Sequence
  source: /note="Description of Artificial Sequence: Synthetic primer"
ccctgggctctgtaaagaa

SEQ ID NO: 2 - DNA, 24 bp, Artificial Sequence
  source: /note="Description of Artificial Sequence: Synthetic primer"
atcagagcttaaactgggaagctg

SEQ ID NO: 3 - DNA, 23 bp, Artificial Sequence
  source: /note="Description of Artificial Sequence: Synthetic primer"
acagtaactgccttcatagatag

SEQ ID NO: 4 - DNA, 22 bp, Artificial Sequence
  source: /note="Description of Artificial Sequence: Synthetic primer"
gtgtcagaccctgttctaagta

SEQ ID NO: 5 - DNA, 30 bp, Artificial Sequence
  source: /note="Description of Artificial Sequence: Synthetic primer"
tgattttcctctttggtatccttatgtaat

SEQ ID NO: 6 - DNA, 28 bp, Artificial Sequence
  source: /note="Description of Artificial Sequence: Synthetic primer"
acaacatttgtatctttatctgtatcct

SEQ ID NO: 7 - DNA, 27 bp, Artificial Sequence
  source: /note="Description of Artificial Sequence: Synthetic primer"
tttgtatttcatgtgtacattcgtatc

SEQ ID NO: 8 - DNA, 28 bp, Artificial Sequence
  source: /note="Description of Artificial Sequence: Synthetic primer"
acctatcctgtagattattttcactgtg

SEQ ID NO: 9 - DNA, 24 bp, Artificial Sequence
  source: /note="Description of Artificial Sequence: Synthetic primer"
ctctgagtgacaaattgagacctt

SEQ ID NO: 10 - DNA, 25 bp, Artificial Sequence
  source: /note="Description of Artificial Sequence: Synthetic primer"
ttaacttctctggtgtgtggagatg

SEQ ID NO: 11 - DNA, 20 bp, Artificial Sequence
  source: /note="Description of Artificial Sequence: Synthetic primer"
tttggtgcacccattacccg

SEQ ID NO: 12 - DNA, 20 bp, Artificial Sequence
  source: /note="Description of Artificial Sequence: Synthetic primer"
aggaggttgaggctgcaaaa

SEQ ID NO: 13 - DNA, 35 bp, Artificial Sequence
  source: /note="Description of Artificial Sequence: Synthetic primer"
caccaaatattggtaattaaatgtttactatagac

SEQ ID NO: 14 - DNA, 25 bp, Artificial Sequence
  source: /note="Description of Artificial Sequence: Synthetic primer"
taaagggtatgatagaacacttgtc

SEQ ID NO: 15 - DNA, 21 bp, Artificial Sequence
  source: /note="Description of Artificial Sequence: Synthetic primer"
caaaggcagatcccaagctct

SEQ ID NO: 16 - DNA, 21 bp, Artificial Sequence
  source: /note="Description of Artificial Sequence: Synthetic primer"
tgtgtgtgcatctgtaagcat

SEQ ID NO: 17 - DNA, 20 bp, Artificial Sequence
  source: /note="Description of Artificial Sequence: Synthetic primer"
tggtgtgtattccctgtgcc

SEQ ID NO: 18 - DNA, 20 bp, Artificial Sequence
  source: /note="Description of Artificial Sequence: Synthetic primer"
gcagtccaatctgggtgaca

SEQ ID NO: 19 - DNA, 28 bp, Artificial Sequence
  source: /note="Description of Artificial Sequence: Synthetic primer"
ccaatctggtcacaaacatattaatgaa

SEQ ID NO: 20 - DNA, 27 bp, Artificial Sequence
  source: /note="Description of Artificial Sequence: Synthetic primer"
tttcccttgtcttgttattaaaggaac

SEQ ID NO: 21 - DNA, 20 bp, Artificial Sequence
  source: /note="Description of Artificial Sequence: Synthetic primer"
ttcccattggcctgttcctc

SEQ ID NO: 22 - DNA, 20 bp, Artificial Sequence
  source: /note="Description of Artificial Sequence: Synthetic primer"
ctgtacacagggcttccgag

SEQ ID NO: 23 - DNA, 23 bp, Artificial Sequence
  source: /note="Description of Artificial Sequence: Synthetic primer"
gctgagtgatttgtctgtaattg

SEQ ID NO: 24 - DNA, 37 bp, Artificial Sequence
  source: /note="Description of Artificial Sequence: Synthetic primer"
gaactcacagattaaactgtaaccaaaataaaattag

SEQ ID NO: 25 - DNA, 22 bp, Artificial Sequence
  source: /note="Description of Artificial Sequence: Synthetic primer"
caatagtgtgcaaggatgggtg

SEQ ID NO: 26 - DNA, 20 bp, Artificial Sequence
  source: /note="Description of Artificial Sequence: Synthetic primer"
tctgtggttctccagcttac

SEQ ID NO: 27 - DNA, 22 bp, Artificial Sequence
  source: /note="Description of Artificial Sequence: Synthetic primer"
cttagggaaccctcactgaatg

SEQ ID NO: 28 - DNA, 22 bp, Artificial Sequence
  source: /note="Description of Artificial Sequence: Synthetic primer"
gtccttgtcagcgtttatttgc

SEQ ID NO: 29 - DNA, 20 bp, Artificial Sequence
  source: /note="Description of Artificial Sequence: Synthetic primer"
ttgggttgagccataggcag

SEQ ID NO: 30 - DNA, 20 bp, Artificial Sequence
  source: /note="Description of Artificial Sequence: Synthetic primer"
gcatccgtgactctctggac

SEQ ID NO: 31 - DNA, 26 bp, Artificial Sequence
  source: /note="Description of Artificial Sequence: Synthetic primer"
gttatgggacttttctcagtctccat

SEQ ID NO: 32 - DNA, 27 bp, Artificial Sequence
  source: /note="Description of Artificial Sequence: Synthetic primer"
gagactaataggaggtagatagactgg

SEQ ID NO: 33 - DNA, 24 bp, Artificial Sequence
  source: /note="Description of Artificial Sequence: Synthetic primer"
gagactgtattagtaaggcttctc

SEQ ID NO: 34 - DNA, 20 bp, Artificial Sequence
  source: /note="Description of Artificial Sequence: Synthetic primer"
cctggactgagccatgctcc

SEQ ID NO: 35 - DNA, 23 bp, Artificial Sequence
  source: /note="Description of Artificial Sequence: Synthetic primer"
cagtcctgtgttagtcaggattc

SEQ ID NO: 36 - DNA, 22 bp, Artificial Sequence
  source: /note="Description of Artificial Sequence: Synthetic primer"
tcaagggtcaactgtgtgatgt

SEQ ID NO: 37 - DNA, 24 bp, Artificial Sequence
  source: /note="Description of Artificial Sequence: Synthetic primer"
cttctgaaagcttctagtttacct

SEQ ID NO: 38 - DNA, 24 bp, Artificial Sequence
  source: /note="Description of Artificial Sequence: Synthetic primer"
ttgcttatttgtgggggtatttca

SEQ ID NO: 39 - DNA, 29 bp, Artificial Sequence
  source: /note="Description of Artificial Sequence: Synthetic primer"
aagaattctcttatttgggttattaattg

SEQ ID NO: 40 - DNA, 20 bp, Artificial Sequence
  source: /note="Description of Artificial Sequence: Synthetic primer"
aaattgtggacaggtgcggt

SEQ ID NO: 41 - DNA, 34 bp, Artificial Sequence
  source: /note="Description of Artificial Sequence: Synthetic primer"
ccatgtaaaaatacatgcatgtgtttatttatac

SEQ ID NO: 42 - DNA, 35 bp, Artificial Sequence
  source: /note="Description of Artificial Sequence: Synthetic primer"
tgattaaaaagaatgaaggtaaaaatgtgtataac

SEQ ID NO: 43 - DNA, 34 bp, Artificial Sequence
  source: /note="Description of Artificial Sequence: Synthetic primer"
ccaaatgtttatgattaatcttttaaattggagc

SEQ ID NO: 44 - DNA, 26 bp, Artificial Sequence
  source: /note="Description of Artificial Sequence: Synthetic primer"
gtaacaagggctacaggaatcatgag

SEQ ID NO: 45 - DNA, 27 bp, Artificial Sequence
  source: /note="Description of Artificial Sequence: Synthetic primer"
tcatccactgaaatgactgaaaaatag

SEQ ID NO: 46 - DNA, 25 bp, Artificial Sequence
  source: /note="Description of Artificial Sequence: Synthetic primer"
aggtacataacagttcaatagaaag

SEQ ID NO: 47 - DNA, 29 bp, Artificial Sequence
  source: /note="Description of Artificial Sequence: Synthetic primer"
gagttattcagtaagttaaaggattgcag

SEQ ID NO: 48 - DNA, 24 bp, Artificial Sequence
  source: /note="Description of Artificial Sequence: Synthetic primer"
gggagccagtggatttggaaacag

SEQ ID NO: 49 - DNA, 20 bp, Artificial Sequence
  source: /note="Description of Artificial Sequence: Synthetic primer"
gcatggtgaggctgaagtag

SEQ ID NO: 50 - DNA, 25 bp, Artificial Sequence
  source: /note="Description of Artificial Sequence: Synthetic primer"
ctaacctatggtcataacgattttt

SEQ ID NO: 51 - DNA, 30 bp, Artificial Sequence
  source: /note="Description of Artificial Sequence: Synthetic primer"
gatgataagaataatcagtatgtgacttgg

SEQ ID NO: 52 - DNA, 30 bp, Artificial Sequence
  source: /note="Description of Artificial Sequence: Synthetic primer"
ataggttagatagagataggacagatgata

SEQ ID NO: 53 - DNA, 22 bp, Artificial Sequence
  source: /note="Description of Artificial Sequence: Synthetic primer"
ccctaccgctatagtaacttgc

SEQ ID NO: 54 - DNA, 23 bp, Artificial Sequence
  source: /note="Description of Artificial Sequence: Synthetic primer"
cacgtctgtaattccagctccta

SEQ ID NO: 55 - DNA, 25 bp, Artificial Sequence
  source: /note="Description of Artificial Sequence: Synthetic primer"
ggaagcgtgtactagagttcttcag

SEQ ID NO: 56 - DNA, 22 bp, Artificial Sequence
  source: /note="Description of Artificial Sequence: Synthetic primer"
ggacagcctccatatccacatg

SEQ ID NO: 57 - DNA, 23 bp, Artificial Sequence
  source: /note="Description of Artificial Sequence: Synthetic primer"
ttcctactgccccacctttattg

SEQ ID NO: 58 - DNA, 24 bp, Artificial Sequence
  source: /note="Description of Artificial Sequence: Synthetic primer"
tttatggtctcagtgcccctcaga

SEQ ID NO: 59 - DNA, 23 bp, Artificial Sequence
  source: /note="Description of Artificial Sequence: Synthetic primer"
tcataatcacatatcacatgagc

SEQ ID NO: 60 - DNA, 21 bp, Artificial Sequence
  source: /note="Description of Artificial Sequence: Synthetic primer"
aaacagaaccaggggaatgaa

SEQ ID NO: 61 - DNA, 25 bp, Artificial Sequence
  source: /note="Description of Artificial Sequence: Synthetic primer"
tgaaactaaagtcaaatggggctac

SEQ ID NO: 62 - DNA, 24 bp, Artificial Sequence
  source: /note="Description of Artificial Sequence: Synthetic primer"
taaggggtgacacctctctggata

SEQ ID NO: 63 - DNA, 25 bp, Artificial Sequence
  source: /note="Description of Artificial Sequence: Synthetic primer"
cccagcctacatctaccacttcatg

SEQ ID NO: 64 - DNA, 28 bp, Artificial Sequence
  source: /note="Description of Artificial Sequence: Synthetic primer"
ctaatgttcgtatggacctttggaaagc

SEQ ID NO: 65 - DNA, 24 bp, Artificial Sequence
  source: /note="Description of Artificial Sequence: Synthetic primer"
gtctccagtacccagctagcttag

SEQ ID NO: 66 - DNA, 22 bp, Artificial Sequence
  source: /note="Description of Artificial Sequence: Synthetic primer"
tctcccaacctgccctttatca

SEQ ID NO: 67 - DNA, 20 bp, Artificial Sequence
  source: /note="Description of Artificial Sequence: Synthetic primer"
tttgggctgacacagtggct

SEQ ID NO: 68 - DNA, 24 bp, Artificial Sequence
  source: /note="Description of Artificial Sequence: Synthetic primer"
ttgatcaacacaggaggtttgacc

SEQ ID NO: 69 - DNA, 30 bp, Artificial Sequence
  source: /note="Description of Artificial Sequence: Synthetic primer"
tataccactttgatgttgacactagtttac

SEQ ID NO: 70 - DNA, 23 bp, Artificial Sequence
  source: /note="Description of Artificial Sequence: Synthetic primer"
cctgtctatggtctcgattcaat

SEQ ID NO: 71 - DNA, 21 bp, Artificial Sequence
  source: /note="Description of Artificial Sequence: Synthetic primer"
tgcatgacagagggagattct

SEQ ID NO: 72 - DNA, 26 bp, Artificial Sequence
  source: /note="Description of Artificial Sequence: Synthetic primer"
agaggggaaatagtagaatgaggatg

SEQ ID NO: 73 - DNA, 24 bp, Artificial Sequence
  source: /note="Description of Artificial Sequence: Synthetic primer"
gccaaactctattagtcaacgttc

SEQ ID NO: 74 - DNA, 24 bp, Artificial Sequence
  source: /note="Description of Artificial Sequence: Synthetic primer"
ctggttctctagctcacatacagt

SEQ ID NO: 75 - DNA, 28 bp, Artificial Sequence
  source: /note="Description of Artificial Sequence: Synthetic primer"
tttacccctaacaagaaaaaaagaagaa

SEQ ID NO: 76 - DNA, 24 bp, Artificial Sequence
  source: /note="Description of Artificial Sequence: Synthetic primer"
cagtgtgagaagtgtgagaagtgc

SEQ ID NO: 77 - DNA, 21 bp, Artificial Sequence
  source: /note="Description of Artificial Sequence: Synthetic primer"
gacaccatgccaaacaacaac

SEQ ID NO: 78 - DNA, 26 bp, Artificial Sequence
  source: /note="Description of Artificial Sequence: Synthetic primer"
atctatctattccaattacatagtcc

SEQ ID NO: 79 - DNA, 30 bp, Artificial Sequence
  source: /note="Description of Artificial Sequence: Synthetic primer"
tcattatacctacttctgtatccaactctc

SEQ ID NO: 80 - DNA, 26 bp, Artificial Sequence
  source: /note="Description of Artificial Sequence: Synthetic primer"
ggaacacaattatccctgagtagcag

SEQ ID NO: 81 - DNA, 29 bp, Artificial Sequence
  source: /note="Description of Artificial Sequence: Synthetic primer"
ggtagcataatagaaattttatgagtggg

SEQ ID NO: 82 - DNA, 30 bp, Artificial Sequence
  source: /note="Description of Artificial Sequence: Synthetic primer"
gaagacagacttcaatatcacagaacatcg

SEQ ID NO: 83 - DNA, 28 bp, Artificial Sequence
  source: /note="Description of Artificial Sequence: Synthetic primer"
gtgtatctattcattcaatcatacaccc

SEQ ID NO: 84 - DNA, 23 bp, Artificial Sequence
  source: /note="Description of Artificial Sequence: Synthetic primer"
ctccctggttgcaagcaattgcc

SEQ ID NO: 85 - DNA, 26 bp, Artificial Sequence
  source: /note="Description of Artificial Sequence: Synthetic primer"
ccaaaattagtggggaatagttgaac

SEQ ID NO: 86 - DNA, 24 bp, Artificial Sequence
  source: /note="Description of Artificial Sequence: Synthetic primer"
gtcgagatcacaccattgcatttc

SEQ ID NO: 87 - DNA, 24 bp, Artificial Sequence
  source: /note="Description of Artificial Sequence: Synthetic primer"
gcctggcttggaattcttttaccc

SEQ ID NO: 88 - DNA, 35 bp, Artificial Sequence
  source: /note="Description of Artificial Sequence: Synthetic primer"
tttaagtctttaatctatcttgaattaatagattc

SEQ ID NO: 89 - DNA, 28 bp, Artificial Sequence
  source: /note="Description of Artificial Sequence: Synthetic primer"
ctttaagaggagtctgctaaaaggaatg

SEQ ID NO: 90 - DNA, 20 bp, Artificial Sequence
  source: /note="Description of Artificial Sequence: Synthetic primer"
tcaccagaaggttgcaagac

SEQ ID NO: 91 - DNA, 20 bp, Artificial Sequence
  source: /note="Description of Artificial Sequence: Synthetic primer"
tctggcgaagtaacccaaac

SEQ ID NO: 92 - DNA, 21 bp, Artificial Sequence
  source: /note="Description of Artificial Sequence: Synthetic primer"
tcgagtcagttcaccagaagg

SEQ ID NO: 93 - DNA, 17 bp, Artificial Sequence
  source: /note="Description of Artificial Sequence: Synthetic primer"
ggaaccagtgagagccg

SEQ ID NO: 94 - DNA, 19 bp, Artificial Sequence
  source: /note="Description of Artificial Sequence: Synthetic primer"
ctcagagtgctgaacccag

SEQ ID NO: 95 - DNA, 32 bp, Artificial Sequence
  source: /note="Description of Artificial Sequence: Synthetic primer"
gtatttattcatgatcagttcttaactcaacc

SEQ ID NO: 96 - DNA, 41 bp, Artificial Sequence
  source: /note="Description of Artificial Sequence: Synthetic primer"
ctacctaatatttatctatatcattctaattatgtctcttc

SEQ ID NO: 97 - DNA, 28 bp, Artificial Sequence
  source: /note="Description of Artificial Sequence: Synthetic primer"
ctctaaaggttttttttggtggcataag

SEQ ID NO: 98 - DNA, 32 bp, Artificial Sequence
  source: /note="Description of Artificial Sequence: Synthetic primer"
gattaatacaacaaaaatttggtaatctgaaa

SEQ ID NO: 99 - DNA, 26 bp, Artificial Sequence
  source: /note="Description of Artificial Sequence: Synthetic primer"
caacctaagctgaaatgcagatattc

SEQ ID NO: 100 - DNA, 30 bp, Artificial Sequence
  source: /note="Description of Artificial Sequence: Synthetic primer"
gttatgaaacgtaaaatgaatgatgactag

SEQ ID NO: 101 - DNA, 26 bp, Artificial Sequence
  source: /note="Description of Artificial Sequence: Synthetic primer"
gcagtctcatttcctggagatgaagg

SEQ ID NO: 102 - DNA, 21 bp, Artificial Sequence
  source: /note="Description of Artificial Sequence: Synthetic primer"
cttgggctgaggagttcaatc

SEQ ID NO: 103 - DNA, 29 bp, Artificial Sequence
  source: /note="Description of Artificial Sequence: Synthetic primer"
gccagtaagaataaaattacagcatgaag

SEQ ID NO: 104 - DNA, 25 bp, Artificial Sequence
  source: /note="Description of Artificial Sequence: Synthetic primer"
gaataatctaccagcaacaatggct

SEQ ID NO: 105 - DNA, 20 bp, Artificial Sequence
  source: /note="Description of Artificial Sequence: Synthetic primer"
tgcccaatggaatgctctct

SEQ ID NO: 106 - DNA, 33 bp, Artificial Sequence
  source: /note="Description of Artificial Sequence: Synthetic primer"
gctccatctcaaacaacaaaaacacaaaaaatg

SEQ ID NO: 107 - DNA, 23 bp, Artificial Sequence
  source: /note="Description of Artificial Sequence: Synthetic primer"
gggtcattgaacctcatgctctg

SEQ ID NO: 108 - DNA, 25 bp, Artificial Sequence
  source: /note="Description of Artificial Sequence: Synthetic primer"
ccccccaaaattctactgaagtaaa

SEQ ID NO: 109 - DNA, 28 bp, Artificial Sequence
  source: /note="Description of Artificial Sequence: Synthetic primer"
taacaggataaatcacctatctatgtat

SEQ ID NO: 110 - DNA, 23 bp, Artificial Sequence
  source: /note="Description of Artificial Sequence: Synthetic primer"
gctgaggagaatttccaaattta

SEQ ID NO: 111 - DNA, 28 bp, Artificial Sequence
  source: /note="Description of Artificial Sequence: Synthetic primer"
cccgcaaactaactaggataaatctcta

SEQ ID NO: 112 - DNA, 28 bp, Artificial Sequence
  source: /note="Description of Artificial Sequence: Synthetic primer"
cgacatgggaaatgtcagatcataagac

SEQ ID NO: 113 - DNA, 28 bp, Artificial Sequence
  source: /note="Description of Artificial Sequence: Synthetic primer"
ccagggagtgaaaaatccttttatcatc

SEQ ID NO: 114 - DNA, 25 bp, Artificial Sequence
  source: /note="Description of Artificial Sequence: Synthetic primer"
gaggatgaaggttagagccagacct

SEQ ID NO: 115 - DNA, 28 bp, Artificial Sequence
  source: /note="Description of Artificial Sequence: Synthetic primer"
tgtggaataaactgaaggctaaagaaaa

SEQ ID NO: 116 - DNA, 28 bp, Artificial Sequence
  source: /note="Description of Artificial Sequence: Synthetic primer"
caagccctatgccaaggatataacaatg

SEQ ID NO: 117 - DNA, 28 bp, Artificial Sequence
  source: /note="Description of Artificial Sequence: Synthetic primer"
gaggttttactgtattaggagttcccac

SEQ ID NO: 118 - DNA, 28 bp, Artificial Sequence
  source: /note="Description of Artificial Sequence: Synthetic primer"
cagatgtgagatgataatttcgttctcc

SEQ ID NO: 119 - DNA, 26 bp, Artificial Sequence
  source: /note="Description of Artificial Sequence: Synthetic primer"
ttgttcttctccatcccatttcaccc

SEQ ID NO: 120 - DNA, 28 bp, Artificial Sequence
  source: /note="Description of Artificial Sequence: Synthetic primer"
cttgtacattcccttatctgctatgtgg

SEQ ID NO: 121 - DNA, 28 bp, Artificial Sequence
  source: /note="Description of Artificial Sequence: Synthetic primer"
ctctctttggagttttatgtgttgctac

SEQ ID NO: 122 - DNA, 28 bp, Artificial Sequence
  source: /note="Description of Artificial Sequence: Synthetic primer"
ctctgatgatgtgcaagaaaggtaggta

SEQ ID NO: 123 - DNA, 29 bp, Artificial Sequence
  source: /note="Description of Artificial Sequence: Synthetic primer"
tcagactatgttttaaggagactatgagg

SEQ ID NO: 124 - DNA, 28 bp, Artificial Sequence
  source: /note="Description of Artificial Sequence: Synthetic primer"
ctaagtatctaccaatgtgctacgtacc

SEQ ID NO: 125 - DNA, 26 bp, Artificial Sequence
  source: /note="Description of Artificial Sequence: Synthetic primer"
cacgtggatgatatggtttctcaagg

SEQ ID NO: 126 - DNA, 28 bp, Artificial Sequence
  source: /note="Description of Artificial Sequence: Synthetic primer"
agcacctatatattatacctgaaagcat

SEQ ID NO: 127 - DNA, 28 bp, Artificial Sequence
  source: /note="Description of Artificial Sequence: Synthetic primer"
cccatgattttcttgtggtgagaatttc

SEQ ID NO: 128 - DNA, 28 bp, Artificial Sequence
  source: /note="Description of Artificial Sequence: Synthetic primer"
caccctctgtactttaatttgacttccc

SEQ ID NO: 129 - DNA, 27 bp, Artificial Sequence
  source: /note="Description of Artificial Sequence: Synthetic primer"
gtttttcttcattcccatgttgtgtac

SEQ ID NO: 130 - DNA, 26 bp, Artificial Sequence
  source: /note="Description of Artificial Sequence: Synthetic primer"
cactcttctgaatcctggtcaacaac

SEQ ID NO: 131 - DNA, 28 bp, Artificial Sequence
  source: /note="Description of Artificial Sequence: Synthetic primer"
caagttatatcatagagtctacgacccc

SEQ ID NO: 132 - DNA, 28 bp, Artificial Sequence
  source: /note="Description of Artificial Sequence: Synthetic primer"
ctgcaactatcagtctctgcccttattc

SEQ ID NO: 133 - DNA, 28 bp, Artificial Sequence
  source: /note="Description of Artificial Sequence: Synthetic primer"
gatgtgtctcaaactgtttattgtgagg

SEQ ID NO: 134 - DNA, 28 bp, Artificial Sequence
  source: /note="Description of Artificial Sequence: Synthetic primer"
gaactcatttatccagagacctgttctc

SEQ ID NO: 135 - DNA, 28 bp, Artificial Sequence
  source: /note="Description of Artificial Sequence: Synthetic primer"
cataatacaacctgtctttggagttact

SEQ ID NO: 136 - DNA, 28 bp, Artificial Sequence
  source: /note="Description of Artificial Sequence: Synthetic primer"
gtgaccagtagttctatgagcaagtatg

SEQ ID NO: 137 - DNA, 28 bp, Artificial Sequence
  source: /note="Description of Artificial Sequence: Synthetic primer"
ccacattgtatggtttttaggcaccatg

SEQ ID NO: 138 - DNA, 28 bp, Artificial Sequence
  source: /note="Description of Artificial Sequence: Synthetic primer"
ctaataagtgggacagttaagagaaggc

SEQ ID NO: 139 - DNA, 27 bp, Artificial Sequence
  source: /note="Description of Artificial Sequence: Synthetic primer"
caagacaagcgattgaaagaagtggat

SEQ ID NO: 140 - DNA, 28 bp, Artificial Sequence
  source: /note="Description of Artificial Sequence: Synthetic primer"
ccttgtcaatctttctaccagagggtaa

SEQ ID NO: 141 - DNA, 25 bp, Artificial Sequence
  source: /note="Description of Artificial Sequence: Synthetic primer"
gaatcatagcttgtgttggtcaggg

SEQ ID NO: 142 - DNA, 27 bp, Artificial Sequence
  source: /note="Description of Artificial Sequence: Synthetic primer"
gaattacaagtatttgcatcccagcct

SEQ ID NO: 143 - DNA, 28 bp, Artificial Sequence
  source: /note="Description of Artificial Sequence: Synthetic primer"
gaccaacttggctttaacagatgcaaat

SEQ ID NO: 144 - DNA, 28 bp, Artificial Sequence
  source: /note="Description of Artificial Sequence: Synthetic primer"
tccttacctttaagacttttcctatttg

SEQ ID NO: 145 - DNA, 28 bp, Artificial Sequence
  source: /note="Description of Artificial Sequence: Synthetic primer"
cattatctcgtcatacttccctgtcttg

SEQ ID NO: 146 - DNA, 28 bp, Artificial Sequence
  source: /note="Description of Artificial Sequence: Synthetic primer"
gcatcaaattcaccagtgaaattattga

SEQ ID NO: 147 - DNA, 28 bp, Artificial Sequence
  source: /note="Description of Artificial Sequence: Synthetic primer"
atgagtacattattcaactgttttggag

SEQ ID NO: 148 - DNA, 28 bp, Artificial Sequence
  source: /note="Description of Artificial Sequence: Synthetic primer"
cagccatgttgtaaacatttttacggtc

SEQ ID NO: 149 - DNA, 28 bp, Artificial Sequence
  source: /note="Description of Artificial Sequence: Synthetic primer"
gcacattctaagaactggtgattctatc

SEQ ID NO: 150 - DNA, 28 bp, Artificial Sequence
  source: /note="Description of Artificial Sequence: Synthetic primer"
gctagaaaaagctgagatagctgtgaag

SEQ ID NO: 151 - DNA, 26 bp, Artificial Sequence
  source: /note="Description of Artificial Sequence: Synthetic primer"
ccttgaagctcattctttgttgtccc

SEQ ID NO: 152 - DNA, 28 bp, Artificial Sequence
  source: /note="Description of Artificial Sequence: Synthetic primer"
ctggacaccagaccaaaaacaaataacc

SEQ ID NO: 153 - DNA, 27 bp, Artificial Sequence
  source: /note="Description of Artificial Sequence: Synthetic primer"
gtaattagagggcagtgaggcttttaa

SEQ ID NO: 154 - DNA, 28 bp, Artificial Sequence
  source: /note="Description of Artificial Sequence: Synthetic primer"
ctccagaagctactgggatattaattag

SEQ ID NO: 155 - DNA, 28 bp, Artificial Sequence
  source: /note="Description of Artificial Sequence: Synthetic primer"
tgagccaaatcagcaatataataggact

SEQ ID NO: 156 - DNA, 28 bp, Artificial Sequence
  source: /note="Description of Artificial Sequence: Synthetic primer"
cctagaaccacaattatctgtctttggc

SEQ ID NO: 157 - DNA, 28 bp, Artificial Sequence
  source: /note="Description of Artificial Sequence: Synthetic primer"
ccattgattctctacagttctgcaggta

SEQ ID NO: 158 - DNA, 28 bp, Artificial Sequence
  source: /note="Description of Artificial Sequence: Synthetic primer"
ctccacactttatacaggtgaaatctga

SEQ ID NO: 159 - DNA, 28 bp, Artificial Sequence
  source: /note="Description of Artificial Sequence: Synthetic primer"
catttttctctccttctgtctcaccttc

SEQ ID NO: 160 - DNA, 28 bp, Artificial Sequence
  source: /note="Description of Artificial Sequence: Synthetic primer"
gcttctctttcccttatgtatctctctc

SEQ ID NO: 161 - DNA, 28 bp, Artificial Sequence
  source: /note="Description of Artificial Sequence: Synthetic primer"
ggcttttgaagaaaaacactaacctgtc

SEQ ID NO: 162 - DNA, 26 bp, Artificial Sequence
  source: /note="Description of Artificial Sequence: Synthetic primer"
cacctatgggctcttcttatttctcc

SEQ ID NO: 163 - DNA, 28 bp, Artificial Sequence
  source: /note="Description of Artificial Sequence: Synthetic primer"
catttgatagccatttgggttgtttcca

SEQ ID NO: 164 - DNA, 28 bp, Artificial Sequence
  source: /note="Description of Artificial Sequence: Synthetic primer"
ccatcacactatcctgacatgaacaaat

SEQ ID NO: 165 - DNA, 26 bp, Artificial Sequence
  source: /note="Description of Artificial Sequence: Synthetic primer"
gaagatttgcatcccagtgaaagcac

SEQ ID NO: 166 - DNA, 28 bp, Artificial Sequence
  source: /note="Description of Artificial Sequence: Synthetic primer"
gcacttcataaagaatcagtcaggatgc

SEQ ID NO: 167 - DNA, 28 bp, Artificial Sequence
  source: /note="Description of Artificial Sequence: Synthetic primer"
ggagaatcaggaaatagtcacttcctac

SEQ ID NO: 168 - DNA, 28 bp, Artificial Sequence
  source: /note="Description of Artificial Sequence: Synthetic primer"
catttgaccttctagccaaatgaagtac

SEQ ID NO: 169 - DNA, 28 bp, Artificial Sequence
  source: /note="Description of Artificial Sequence: Synthetic primer"
ggaatttctgagaataacattgcctctc

SEQ ID NO: 170 - DNA, 28 bp, Artificial Sequence
  source: /note="Description of Artificial Sequence: Synthetic primer"
catatgttgggggagctaaacctaatga

SEQ ID NO: 171 - DNA, 27 bp, Artificial Sequence
  source: /note="Description of Artificial Sequence: Synthetic primer"
cactgtgaccacagcatcttttaactc

SEQ ID NO: 172 - DNA, 28 bp, Artificial Sequence
  source: /note="Description of Artificial Sequence: Synthetic primer"
gggtaaagaaatattcagcacatccaaa

SEQ ID NO: 173 - DNA, 28 bp, Artificial Sequence
  source: /note="Description of Artificial Sequence: Synthetic primer"
gagtatcccttatctaaaatgctggtcc

SEQ ID NO: 174 - DNA, 28 bp, Artificial Sequence
  source: /note="Description of Artificial Sequence: Synthetic primer"
ctttttctcttaccggaacttcaacgac

SEQ ID NO: 175 - DNA, 28 bp, Artificial Sequence
  source: /note="Description of Artificial Sequence: Synthetic primer"
cctcattaatatgaccaaggctcctctg

SEQ ID NO: 176 - DNA, 28 bp, Artificial Sequence
  source: /note="Description of Artificial Sequence: Synthetic primer"
tgactctaattggggatgtggtaattag

SEQ ID NO: 177 - DNA, 25 bp, Artificial Sequence
  source: /note="Description of Artificial Sequence: Synthetic primer"
gacctaacctggagaaaaccggaga

SEQ ID NO: 178 - DNA, 28 bp, Artificial Sequence
  source: /note="Description of Artificial Sequence: Synthetic primer"
gtttctcttctctgaacctttgtctcag

SEQ ID NO: 179 - DNA, 28 bp, Artificial Sequence
  source: /note="Description of Artificial Sequence: Synthetic primer"
gcaaacacacaaagataggttcgagttt

SEQ ID NO: 180 - DNA, 28 bp, Artificial Sequence
  source: /note="Description of Artificial Sequence: Synthetic primer"
catatcaagtgctttctgttgacatttg

SEQ ID NO: 181 - DNA, 28 bp, Artificial Sequence
  source: /note="Description of Artificial Sequence: Synthetic primer"
ctgaaaagtgctacgtaagaggtcattg

SEQ ID NO: 182 - DNA, 25 bp, Artificial Sequence
  source: /note="Description of Artificial Sequence: Synthetic primer"
catctgagtgtgagaagagcctcaa

SEQ ID NO: 183 - DNA, 28 bp, Artificial Sequence
  source: /note="Description of Artificial Sequence: Synthetic primer"
cccagcaaaaacttcttttctccagtaa

SEQ ID NO: 184 - DNA, 28 bp, Artificial Sequence
  source: /note="Description of Artificial Sequence: Synthetic primer"
gctaggaaagttttctctctggttcaca

SEQ ID NO: 185 - DNA, 27 bp, Artificial Sequence
  source: /note="Description of Artificial Sequence: Synthetic primer"
gaatatctatgagcaggcagttagcag

SEQ ID NO: 186 - DNA, 28 bp, Artificial Sequence
  source: /note="Description of Artificial Sequence: Synthetic primer"
ctaatcagtgtcactatgtgtgagctat

SEQ ID NO: 187 - DNA, 28 bp, Artificial Sequence
  source: /note="Description of Artificial Sequence: Synthetic primer"
catcatacagactcaaggagcttagctg

SEQ ID NO: 188 - DNA, 28 bp, Artificial Sequence
  source: /note="Description of Artificial Sequence: Synthetic primer"
ctttccaagccttggaaaacacagaaaa

SEQ ID NO: 189 - DNA, 27 bp, Artificial Sequence
  source: /note="Description of Artificial Sequence: Synthetic primer"
gtaccttataaatcacggagtgcagac

SEQ ID NO: 190 - DNA, 27 bp, Artificial Sequence
  source: /note="Description of Artificial Sequence: Synthetic primer"
caagtggtaagagatgactgaggtcaa

SEQ ID NO: 191 - DNA, 28 bp, Artificial Sequence
  source: /note="Description of Artificial Sequence: Synthetic primer"
cttcttctcttagaaggacactggtcag

SEQ ID NO: 192 - DNA, 27 bp, Artificial Sequence
  source: /note="Description of Artificial Sequence: Synthetic primer"
gttatggaggattggtaagaaccagag

SEQ ID NO: 193 - DNA, 28 bp, Artificial Sequence
  source: /note="Description of Artificial Sequence: Synthetic primer"
gagctgtttaagggtaaaggggtagtta

SEQ ID NO: 194 - DNA, 28 bp, Artificial Sequence
  source: /note="Description of Artificial Sequence: Synthetic primer"
gcagacaaaaccatgacaatgatcttag

SEQ ID NO: 195 - DNA, 28 bp, Artificial Sequence
  source: /note="Description of Artificial Sequence: Synthetic primer"
cccatgatgaaacagtttgcactaaatg

SEQ ID NO: 196 - DNA, 27 bp, Artificial Sequence
  source: /note="Description of Artificial Sequence: Synthetic primer"
ctcaattttcttgtccctgctttcatg

SEQ ID NO: 197 - DNA, 28 bp, Artificial Sequence
  source: /note="Description of Artificial Sequence: Synthetic primer"
ttagaaattccagatagagctaaaactg

SEQ ID NO: 198 - DNA, 25 bp, Artificial Sequence
  source: /note="Description of Artificial Sequence: Synthetic primer"
gttaggaaaagaacccaggtgtttt

SEQ ID NO: 199 - DNA, 27 bp, Artificial Sequence
  source: /note="Description of Artificial Sequence: Synthetic primer"
gcaaaagtaaatacaaaggcatacttt

SEQ ID NO: 200 - DNA, 28 bp, Artificial Sequence
  source: /note="Description of Artificial Sequence: Synthetic primer"
caatgcaaaagaaaggtccttactcgac

SEQ ID NO: 201 - DNA, 28 bp, Artificial Sequence
  source: /note="Description of Artificial Sequence: Synthetic primer"
catttctaaactctaaaacaaacatttg

SEQ ID NO: 202 - DNA, 28 bp, Artificial Sequence
  source: /note="Description of Artificial Sequence: Synthetic primer"
ggtccttaacctattaaattttaatgag

SEQ ID NO: 203 - DNA, 28 bp, Artificial Sequence
  source: /note="Description of Artificial Sequence: Synthetic primer"
gactttcaatttatgtcagcatttaaaa

SEQ ID NO: 204 - DNA, 27 bp, Artificial Sequence
  source: /note="Description of Artificial Sequence: Synthetic primer"
cctcttggttgcattggattctcattg

SEQ ID NO: 205 - DNA, 27 bp, Artificial Sequence
  source: /note="Description of Artificial Sequence: Synthetic primer"
tctccatgaaacttgggttaattttgc

SEQ ID NO: 206 - DNA, 25 bp, Artificial Sequence
  source: /note="Description of Artificial Sequence: Synthetic primer"
tgtctggaagttcgtcaaattgcag

SEQ ID NO: 207 - DNA, 28 bp, Artificial Sequence
  source: /note="Description of Artificial Sequence: Synthetic primer"
gtagcataaaacattccaaaaattcaat

SEQ ID NO: 208 - DNA, 30 bp, Artificial Sequence
  source: /note="Description of Artificial Sequence: Synthetic primer"
tgctttaaagatacaggttatctgtattac

SEQ ID NO: 209 - DNA, 26 bp, Artificial Sequence
  source: /note="Description of Artificial Sequence: Synthetic primer"
ctctccgttactttcttcctgccttt

SEQ ID NO: 210 - DNA, 26 bp, Artificial Sequence
  source: /note="Description of Artificial Sequence: Synthetic primer"
gatcctgagattcacctctagtccct

SEQ ID NO: 211 - DNA, 26 bp, Artificial Sequence
  source: /note="Description of Artificial Sequence: Synthetic primer"
ccgtaccaggtacctagctatgtact

SEQ ID NO: 212 - DNA, 27 bp, Artificial Sequence
  source: /note="Description of Artificial Sequence: Synthetic primer"
ctttctgttttgtccatctgaaattct

SEQ ID NO: 213 - DNA, 27 bp, Artificial Sequence
  source: /note="Description of Artificial Sequence: Synthetic primer"
caaagttaagtatcaccatccagctgg

SEQ ID NO: 214 - DNA, 28 bp, Artificial Sequence
  source: /note="Description of Artificial Sequence: Synthetic primer"
atagggatagctgataagaaacatgacc

SEQ ID NO: 215 - DNA, 25 bp, Artificial Sequence
  source: /note="Description of Artificial Sequence: Synthetic primer"
cttaataagacgctgcatctgccca

SEQ ID NO: 216 - DNA, 28 bp, Artificial Sequence
  source: /note="Description of Artificial Sequence: Synthetic primer"
tccaggagacatttgttcatataagtga

SEQ ID NO: 217 - DNA, 28 bp, Artificial Sequence
  source: /note="Description of Artificial Sequence: Synthetic primer"
agacacttttcagtatccatttagaaac

SEQ ID NO: 218 - DNA, 25 bp, Artificial Sequence
  source: /note="Description of Artificial Sequence: Synthetic primer"
gtttcacatgtgcatgcttttgggt

SEQ ID NO: 219 - DNA, 26 bp, Artificial Sequence
  source: /note="Description of Artificial Sequence: Synthetic primer"
ccaaagctattctctcttttgggtgc

SEQ ID NO: 220 - DNA, 27 bp, Artificial Sequence
  source: /note="Description of Artificial Sequence: Synthetic primer"
gaaagttcacttcagatgttcaaagcc

SEQ ID NO: 221 - DNA, 26 bp, Artificial Sequence
  source: /note="Description of Artificial Sequence: Synthetic primer"
gggtttcagtctgcaacaagatcttg

SEQ ID NO: 222 - DNA, 28 bp, Artificial Sequence
  source: /note="Description of Artificial Sequence: Synthetic primer"
tggagatcaatatttagccttaacatat

SEQ ID NO: 223 - DNA, 28 bp, Artificial Sequence
  source: /note="Description of Artificial Sequence: Synthetic primer"
gactgtttctcatcctgttattatttgt

SEQ ID NO: 224 - DNA, 25 bp, Artificial Sequence
  source: /note="Description of Artificial Sequence: Synthetic primer"
aacacacagaaacatcaagctgagc

SEQ ID NO: 225 - DNA, 27 bp, Artificial Sequence
  source: /note="Description of Artificial Sequence: Synthetic primer"
ttcctgacattctccttcttctatctg

SEQ ID NO: 226 - DNA, 26 bp, Artificial Sequence
  source: /note="Description of Artificial Sequence: Synthetic primer"
tatgacgcctggattttcacaacaac

SEQ ID NO: 227 - DNA, 28 bp, Artificial Sequence
  source: /note="Description of Artificial Sequence: Synthetic primer"
cagagactatggatggtatttaggtcaa

SEQ ID NO: 228 - DNA, 25 bp, Artificial Sequence
  source: /note="Description of Artificial Sequence: Synthetic primer"
actttgtgtggctgagagagagaaa

SEQ ID NO: 229 - DNA, 30 bp, Artificial Sequence
  source: /note="Description of Artificial Sequence: Synthetic primer"
tgagtgttctctgtattttcttactctaag

SEQ ID NO: 230 - DNA, 27 bp, Artificial Sequence
  source: /note="Description of Artificial Sequence: Synthetic primer"
atttttggtcattgttgacacttcacc

SEQ ID NO: 231 - DNA, 25 bp, Artificial Sequence
  source: /note="Description of Artificial Sequence: Synthetic primer"
ggtgttagggagacaggcatgaatg

SEQ ID NO: 232 - DNA, 26 bp, Artificial Sequence
  source: /note="Description of Artificial Sequence: Synthetic primer"
tgaaacttttcaactctcctaccgcc

SEQ ID NO: 233 - DNA, 28 bp, Artificial Sequence
  source: /note="Description of Artificial Sequence: Synthetic primer"
gttaaaattgccactaattatgtgtttt

SEQ ID NO: 234 - DNA, 27 bp, Artificial Sequence
  source: /note="Description of Artificial Sequence: Synthetic primer"
aactgatcctatgcagcaagatctttg

SEQ ID NO: 235 - DNA, 27 bp, Artificial Sequence
  source: /note="Description of Artificial Sequence: Synthetic primer"
gatgcttgcaaacaaagactgaaaagg

SEQ ID NO: 236 - DNA, 28 bp, Artificial Sequence
  source: /note="Description of Artificial Sequence: Synthetic primer"
gtctgtgtgtcctctgagatgatgaatg

SEQ ID NO: 237 - DNA, 26 bp, Artificial Sequence
  source: /note="Description of Artificial Sequence: Synthetic primer"
gggaggaagaaaacagagagtcttga

SEQ ID NO: 238 - DNA, 28 bp, Artificial Sequence
  source: /note="Description of Artificial Sequence: Synthetic primer"
agtttgttggcttcttttgagaagtatc

SEQ ID NO: 239 - DNA, 28 bp, Artificial Sequence
  source: /note="Description of Artificial Sequence: Synthetic primer"
ggcagatgaagtagtagatatctggctg

SEQ ID NO: 240 - DNA, 27 bp, Artificial Sequence
  source: /note="Description of Artificial Sequence: Synthetic primer"
gttcagtgtcaattttgaccagatatt

SEQ ID NO: 241 - DNA, 28 bp, Artificial Sequence
  source: /note="Description of Artificial Sequence: Synthetic primer"
agacataggacacaccattttattgtct

SEQ ID NO: 242 - DNA, 28 bp, Artificial Sequence
  source: /note="Description of Artificial Sequence: Synthetic primer"
tcaaaatatttggctaaactattgccgg

SEQ ID NO: 243 - DNA, 31 bp, Artificial Sequence
  source: /note="Description of Artificial Sequence: Synthetic primer"
ctggagttattaataaattggattatatagc

SEQ ID NO: 244 - DNA, 27 bp, Artificial Sequence
  source: /note="Description of Artificial Sequence: Synthetic primer"
ttacctgttttccttttgtgattccac

SEQ ID NO: 245 - DNA, 26 bp, Artificial Sequence
  source: /note="Description of Artificial Sequence: Synthetic primer"
accaagtcaagagctctgagagacat

SEQ ID NO: 246 - DNA, 28 bp, Artificial Sequence
  source: /note="Description of Artificial Sequence: Synthetic primer"
acagtgaatgatattcagaatattgtgc

SEQ ID NO: 247 - DNA, 28 bp, Artificial Sequence
  source: /note="Description of Artificial Sequence: Synthetic primer"
gaacaaggtcaagatatcagctttcacc

SEQ ID NO: 248 - DNA, 26 bp, Artificial Sequence
  source: /note="Description of Artificial Sequence: Synthetic primer"
aggtcatacaatgaatggtgtgatgt

SEQ ID NO: 249 - DNA, 27 bp, Artificial Sequence
  source: /note="Description of Artificial Sequence: Synthetic primer"
atccacccatgagaaatatatccacaa

SEQ ID NO: 250 - DNA, 31 bp, Artificial Sequence
  source: /note="Description of Artificial Sequence: Synthetic primer"
acaattcaaattaatgtaaaaactgcaagtg

SEQ ID NO: 251 - DNA, 25 bp, Artificial Sequence
  source: /note="Description of Artificial Sequence: Synthetic primer"
tagttctagtgtgggatctgactcc

SEQ ID NO: 252 - DNA, 27 bp, Artificial Sequence
  source: /note="Description of Artificial Sequence: Synthetic primer"
gaacatctgttcaggtttctctccatc

SEQ ID NO: 253 - DNA, 27 bp, Artificial Sequence
  source: /note="Description of Artificial Sequence: Synthetic primer"
gaaaggactaaattgttgaacactggt

SEQ ID NO: 254 - DNA, 25 bp, Artificial Sequence
  source: /note="Description of Artificial Sequence: Synthetic primer"
tgtgtgttttaaagccaggtttgtt

SEQ ID NO: 255 - DNA, 25 bp, Artificial Sequence
  source: /note="Description of Artificial Sequence: Synthetic primer"
gatggactggaactgaggattttca

SEQ ID NO: 256 - DNA, 29 bp, Artificial Sequence
  source: /note="Description of Artificial Sequence: Synthetic primer"
agctttagaaaggcatatcgtattaactg

SEQ ID NO: 257 - DNA, 25 bp, Artificial Sequence
  source: /note="Description of Artificial Sequence: Synthetic primer"
ttatagtgagtaaaggacaggcccc

SEQ ID NO: 258 - DNA, 29 bp, Artificial Sequence
  source: /note="Description of Artificial Sequence: Synthetic primer"
acacatctgttgacagtaatgaaatatcc

SEQ ID NO: 259 - DNA, 28 bp, Artificial Sequence
  source: /note="Description of Artificial Sequence: Synthetic primer"
gtttaaacttggataccatccccaagac

SEQ ID NO: 260 - DNA, 25 bp, Artificial Sequence
  source: /note="Description of Artificial Sequence: Synthetic primer"
atgagattgctgggagatgcagatg

SEQ ID NO: 261 - DNA, 26 bp, Artificial Sequence
  source: /note="Description of Artificial Sequence: Synthetic primer"
cacatttccctcttgcggttacatac

SEQ ID NO: 262 - DNA, 25 bp, Artificial Sequence
  source: /note="Description of Artificial Sequence: Synthetic primer"
gacaagcctcgcttgagttttcttt

SEQ ID NO: 263 - DNA, 25 bp, Artificial Sequence
  source: /note="Description of Artificial Sequence: Synthetic primer"
tgtgagagtgtcaccgaattcaacg

SEQ ID NO: 264 - DNA, 27 bp, Artificial Sequence
  source: /note="Description of Artificial Sequence: Synthetic primer"
aaatagcaatggctcgtctatggttag

SEQ ID NO: 265 - DNA, 27 bp, Artificial Sequence
  source: /note="Description of Artificial Sequence: Synthetic primer"
tgctaagtaaggtgagtggtataatca

SEQ ID NO: 266 - DNA, 27 bp, Artificial Sequence
  source: /note="Description of Artificial Sequence: Synthetic primer"
ataaatatgatgtggctactccctcat

SEQ ID NO: 267 - DNA, 29 bp, Artificial Sequence
  source: /note="Description of Artificial Sequence: Synthetic primer"
gctacacctccatagtaataatgtaagag

SEQ ID NO: 268 - DNA, 26 bp, Artificial Sequence
  source: /note="Description of Artificial Sequence: Synthetic primer"
tgaagcagctagagaactctgtacgt

SEQ ID NO: 269 - DNA, 31 bp, Artificial Sequence
  source: /note="Description of Artificial Sequence: Synthetic primer"
ttttgtctctgttatattagtcacctatctc

SEQ ID NO: 270 - DNA, 26 bp, Artificial Sequence
  source: /note="Description of Artificial Sequence: Synthetic primer"
atagccctgcattcaaatcccaagtg

SEQ ID NO: 271 - DNA, 26 bp, Artificial Sequence
  source: /note="Description of Artificial Sequence: Synthetic primer"
tccatttttataccactgcactgaag

SEQ ID NO: 272 - DNA, 28 bp, Artificial Sequence
  source: /note="Description of Artificial Sequence: Synthetic primer"
gcagtaaaacattttcatcaaatttcca

SEQ ID NO: 273 - DNA, 27 bp, Artificial Sequence
  source: /note="Description of Artificial Sequence: Synthetic primer"
tctgggtgcaaactagctgaatatcag

SEQ ID NO: 274 - DNA, 27 bp, Artificial Sequence
  source: /note="Description of Artificial Sequence: Synthetic primer"
gaaaatctggaggcaattcatgatgcc

SEQ ID NO: 275 - DNA, 26 bp, Artificial Sequence
  source: /note="Description of Artificial Sequence: Synthetic primer"
atacaatgatgatcacacgggaccct

SEQ ID NO: 276 - DNA, 27 bp, Artificial Sequence
  source: /note="Description of Artificial Sequence: Synthetic primer"
ccatgaagatggagtcaacattttaca

SEQ ID NO: 277 - DNA, 26 bp, Artificial Sequence
  source: /note="Description of Artificial Sequence: Synthetic primer"
tcctaacccctagtacgttagatgtg

SEQ ID NO: 278 - DNA, 25 bp, Artificial Sequence
  source: /note="Description of Artificial Sequence: Synthetic primer"
gaggtgatttctgtgaggaacgtcg

SEQ ID NO: 279 - DNA, 28 bp, Artificial Sequence
  source: /note="Description of Artificial Sequence: Synthetic primer"
gtacattcacttaacaggctctctttcc

SEQ ID NO: 280 - DNA, 25 bp, Artificial Sequence
  source: /note="Description of Artificial Sequence: Synthetic primer"
aattcatgagctggtgtccaaggag

SEQ ID NO: 281 - DNA, 29 bp, Artificial Sequence
  source: /note="Description of Artificial Sequence: Synthetic primer"
ataacagtctccagagtatattagcttag

SEQ ID NO: 282 - DNA, 25 bp, Artificial Sequence
  source: /note="Description of Artificial Sequence: Synthetic primer"
gttcctctgggatgcaacatgagag

SEQ ID NO: 283 - DNA, 28 bp, Artificial Sequence
  source: /note="Description of Artificial Sequence: Synthetic primer"
gaaaggatgaagagggtggatattggag

SEQ ID NO: 284 - DNA, 28 bp, Artificial Sequence
  source: /note="Description of Artificial Sequence: Synthetic primer"
ccaaacctcatcatctcttacctggatt

SEQ ID NO: 285 - DNA, 28 bp, Artificial Sequence
  source: /note="Description of Artificial Sequence: Synthetic primer"
gtccaaagtcaagtgcaagtatagttgg

SEQ ID NO: 286 - DNA, 28 bp, Artificial Sequence
  source: /note="Description of Artificial Sequence: Synthetic primer"
acaatcttttctgaatctgaacagcttc

SEQ ID NO: 287 - DNA, 28 bp, Artificial Sequence
  source: /note="Description of Artificial Sequence: Synthetic primer"
caaaggaaggcatttcctaatgatcttc

SEQ ID NO: 288 - DNA, 28 bp, Artificial Sequence
  source: /note="Description of Artificial Sequence: Synthetic primer"
ctttgctttgcttttcttcttcagggaa

SEQ ID NO: 289 - DNA, 28 bp, Artificial Sequence
  source: /note="Description of Artificial Sequence: Synthetic primer"
ctgcttcaagtgtatataaactcacagt

SEQ ID NO: 290 - DNA, 28 bp, Artificial Sequence
  source: /note="Description of Artificial Sequence: Synthetic primer"
cctaggaaagcagtaactaattcaggag

SEQ ID NO: 291 - DNA, 28 bp, Artificial Sequence
  source: /note="Description of Artificial Sequence: Synthetic primer"
gcaatttgttcacttttagtttcgtagc

SEQ ID NO: 292 - DNA, 28 bp, Artificial Sequence
  source: /note="Description of Artificial Sequence: Synthetic primer"
ggcctaatatgcatgtgttcatgtctct

SEQ ID NO: 293 - DNA, 28 bp, Artificial Sequence
  source: /note="Description of Artificial Sequence: Synthetic primer"
cagagtttctcatctacgaaagaggagt

SEQ ID NO: 294 - DNA, 26 bp, Artificial Sequence
  source: /note="Description of Artificial Sequence: Synthetic primer"
atcctagacctccaggtggaatgatc

SEQ ID NO: 295 - DNA, 28 bp, Artificial Sequence
  source: /note="Description of Artificial Sequence: Synthetic primer"
cttggctgtctcaatattttggagtaag

SEQ ID NO: 296 - DNA, 28 bp, Artificial Sequence
  source: /note="Description of Artificial Sequence: Synthetic primer"
gagtaaatgagctgtggtttctctctta

SEQ ID NO: 297 - DNA, 28 bp, Artificial Sequence
  source: /note="Description of Artificial Sequence: Synthetic primer"
ctttccatgtggaccctttaacattcag

SEQ ID NO: 298 - DNA, 28 bp, Artificial Sequence
  source: /note="Description of Artificial Sequence: Synthetic primer"
gcatagtgagctgttgatagagcttttg

SEQ ID NO: 299 - DNA, 28 bp, Artificial Sequence
  source: /note="Description of Artificial Sequence: Synthetic primer"
ctagaacaaaatcattggctctcctagt

SEQ ID NO: 300 - DNA, 27 bp, Artificial Sequence
  source: /note="Description of Artificial Sequence: Synthetic primer"
gtctggtgagtactggctgaatgtaaa

SEQ ID NO: 301 - DNA, 28 bp, Artificial Sequence
  source: /note="Description of Artificial Sequence: Synthetic primer"
ccagaggatgctgctaaacattctacaa

SEQ ID NO: 302 - DNA, 28 bp, Artificial Sequence
  source: /note="Description of Artificial Sequence: Synthetic primer"
gctcatgcctggaattcacctttatttt

SEQ ID NO: 303 - DNA, 28 bp, Artificial Sequence
  source: /note="Description of Artificial Sequence: Synthetic primer"
ctaactagacatttgggccaccttactt

SEQ ID NO: 304 - DNA, 28 bp, Artificial Sequence
  source: /note="Description of Artificial Sequence: Synthetic primer"
gtctatggtgcctatagaatgtacaggt

SEQ ID NO: 305 - DNA, 28 bp, Artificial Sequence
  source: /note="Description of Artificial Sequence: Synthetic primer"
ccctctcaagtttgtgagcaaatatcac

SEQ ID NO: 306 - DNA, 26 bp, Artificial Sequence
  source: /note="Description of Artificial Sequence: Synthetic primer"
ctctatcttgctgcaatggactttcc

SEQ ID NO: 307 - DNA, 28 bp, Artificial Sequence
  source: /note="Description of Artificial Sequence: Synthetic primer"
cctagaaacagattttgaagggctcttg

SEQ ID NO: 308 - DNA, 25 bp, Artificial Sequence
  source: /note="Description of Artificial Sequence: Synthetic primer"
aaatgaggggcatagggataaggga

SEQ ID NO: 309 - DNA, 28 bp, Artificial Sequence
  source: /note="Description of Artificial Sequence: Synthetic primer"
cctagaaatctgatacgttatcctatga

SEQ ID NO: 310 - DNA, 28 bp, Artificial Sequence
  source: /note="Description of Artificial Sequence: Synthetic primer"
aggagagatatattcaacatgaacccaa

SEQ ID NO: 311 - DNA, 28 bp, Artificial Sequence
  source: /note="Description of Artificial Sequence: Synthetic primer"
gaacatctctgaccagaaatttccagta

SEQ ID NO: 312 - DNA, 28 bp, Artificial Sequence
  source: /note="Description of Artificial Sequence: Synthetic primer"
gtgtagtgaaatccttagacttaggtaa

SEQ ID NO: 313 - DNA, 28 bp, Artificial Sequence
  source: /note="Description of Artificial Sequence: Synthetic primer"
aatacatgaaaaagtaatacatggggca

SEQ ID NO: 314 - DNA, 28 bp, Artificial Sequence
  source: /note="Description of Artificial Sequence: Synthetic primer"
attaaatgtttacttctatctacaagga

SEQ ID NO: 315 - DNA, 28 bp, Artificial Sequence
  source: /note="Description of Artificial Sequence: Synthetic primer"
cattttgtgaaatgcaaagggcaaatct

SEQ ID NO: 316 - DNA, 28 bp, Artificial Sequence
  source: /note="Description of Artificial Sequence: Synthetic primer"
gctgagaggcttaattccatcaagatga

SEQ ID NO: 317 - DNA, 28 bp, Artificial Sequence
  source: /note="Description of Artificial Sequence: Synthetic primer"
cccatcctaaacttagttttatgggcag

SEQ ID NO: 318 - DNA, 27 bp, Artificial Sequence
  source: /note="Description of Artificial Sequence: Synthetic primer"
gtaacacattctctttgggaagctagc

SEQ ID NO: 319 - DNA, 28 bp, Artificial Sequence
  source: /note="Description of Artificial Sequence: Synthetic primer"
cttagcttcagtgaaaatggttcctctc

SEQ ID NO: 320 - DNA, 28 bp, Artificial Sequence
  source: /note="Description of Artificial Sequence: Synthetic primer"
ctttcttagctcctctccatttctcttc

SEQ ID NO: 321 - DNA, 28 bp, Artificial Sequence
  source: /note="Description of Artificial Sequence: Synthetic primer"
gtctatgcagtgcttcactgaggattat

SEQ ID NO: 322 - DNA, 28 bp, Artificial Sequence
  source: /note="Description of Artificial Sequence: Synthetic primer"
ctctatctgctcagagcctgcttaaaag

SEQ ID NO: 323 - DNA, 28 bp, Artificial Sequence
  source: /note="Description of Artificial Sequence: Synthetic primer"
ggaaaggatacagtgttgagcaagatag

SEQ ID NO: 324 - DNA, 28 bp, Artificial Sequence
  source: /note="Description of Artificial Sequence: Synthetic primer"
gccaacttgattctctttcaaatgcttg

SEQ ID NO: 325 - DNA, 25 bp, Artificial Sequence
  source: /note="Description of Artificial Sequence: Synthetic primer"
agatggggtttaccatgtttcccag

SEQ ID NO: 326 - DNA, 28 bp, Artificial Sequence
  source: /note="Description of Artificial Sequence: Synthetic primer"
gtacagtagttagtttccagactgatga

SEQ ID NO: 327 - DNA, 28 bp, Artificial Sequence
  source: /note="Description of Artificial Sequence: Synthetic primer"
gtaaatatctaactgtgtttccctcagt

SEQ ID NO: 328 - DNA, 28 bp, Artificial Sequence
  source: /note="Description of Artificial Sequence: Synthetic primer"
gaaccaaaaggaattaagagactagggg

SEQ ID NO: 329 - DNA, 27 bp, Artificial Sequence
  source: /note="Description of Artificial Sequence: Synthetic primer"
ctgcttttacggcttcttcctttcttc

SEQ ID NO: 330 - DNA, 26 bp, Artificial Sequence
  source: /note="Description of Artificial Sequence: Synthetic primer"
cccacatccttcccatttataggcaa

SEQ ID NO: 331 - DNA, 25 bp, Artificial Sequence
  source: /note="Description of Artificial Sequence: Synthetic primer"
tacatgatcctaagggcagcaggaa

SEQ ID NO: 332 - DNA, 25 bp, Artificial Sequence
  source: /note="Description of Artificial Sequence: Synthetic primer"
gtttggtgcatcctctttctctctc

SEQ ID NO: 333 - DNA, 25 bp, Artificial Sequence
  source: /note="Description of Artificial Sequence: Synthetic primer"
gactgtagtcaccccttctccaaca

SEQ ID NO: 334 - DNA, 31 bp, Artificial Sequence
  source: /note="Description of Artificial Sequence: Synthetic primer"
agagtgaaatacatagaaaagaaacttaaag

SEQ ID NO: 335 - DNA, 28 bp, Artificial Sequence
  source: /note="Description of Artificial Sequence: Synthetic primer"
atttgcgagaaacagataaatattgaag

SEQ ID NO: 336 - DNA, 28 bp, Artificial Sequence
  source: /note="Description of Artificial Sequence: Synthetic primer"
acaggaacaaagaatttgttcttcatgg

SEQ ID NO: 337 - DNA, 25 bp, Artificial Sequence
  source: /note="Description of Artificial Sequence: Synthetic primer"
ccttggattgtctcaggatgttgca

SEQ ID NO: 338 - DNA, 25 bp, Artificial Sequence
  source: /note="Description of Artificial Sequence: Synthetic primer"
ctgggatgtttgttttggctttgtg

SEQ ID NO: 339 - DNA, 30 bp, Artificial Sequence
  source: /note="Description of Artificial Sequence: Synthetic primer"
attggtagtacactaatggatatatgtgag

SEQ ID NO: 340 - DNA, 27 bp, Artificial Sequence
  source: /note="Description of Artificial Sequence: Synthetic primer"
gaataaagtgaggaaaacacggagttg

SEQ ID NO: 341 - DNA, 25 bp, Artificial Sequence
  source: /note="Description of Artificial Sequence: Synthetic primer"
gagagaggcagaaaggagggatgaa

SEQ ID NO: 342 - DNA, 28 bp, Artificial Sequence
  source: /note="Description of Artificial Sequence: Synthetic primer"
tactctgtcttcagtagctgtttcttgg

SEQ ID NO: 343 - DNA, 28 bp, Artificial Sequence
  source: /note="Description of Artificial Sequence: Synthetic primer"
ttagactcaccaagatcaagatgaatgc

SEQ ID NO: 344 - DNA, 29 bp, Artificial Sequence
  source: /note="Description of Artificial Sequence: Synthetic primer"
atctcaataaagctgttcaaaacagaaag

SEQ ID NO: 345 - DNA, 26 bp, Artificial Sequence
  source: /note="Description of Artificial Sequence: Synthetic primer"
taaagaaaatgccatgggctgtaccc

SEQ ID NO: 346 - DNA, 26 bp, Artificial Sequence
  source: /note="Description of Artificial Sequence: Synthetic primer"
attgtgcagcagaacagagtgtagtg

SEQ ID NO: 347 - DNA, 28 bp, Artificial Sequence
  source: /note="Description of Artificial Sequence: Synthetic primer"
attctttgcatagctcacgaaatttccc

SEQ ID NO: 348 - DNA, 26 bp, Artificial Sequence
  source: /note="Description of Artificial Sequence: Synthetic primer"
aaaatgagacctcgtatctttgcagc

SEQ ID NO: 349 - DNA, 26 bp, Artificial Sequence
  source: /note="Description of Artificial Sequence: Synthetic primer"
aaatgcagaactgccaaaagaaaccc

SEQ ID NO: 350 - DNA, 25 bp, Artificial Sequence
  source: /note="Description of Artificial Sequence: Synthetic primer"
gagaatctgtgaatgccagggtctg

SEQ ID NO: 351 - DNA, 27 bp, Artificial Sequence
  source: /note="Description of Artificial Sequence: Synthetic primer"
atggattcatgtttcagacatctaatt

SEQ ID NO: 352 - DNA, 28 bp, Artificial Sequence
  source: /note="Description of Artificial Sequence: Synthetic primer"
atcactagaaagaaaagagttcctattc

SEQ ID NO: 353 - DNA, 27 bp, Artificial Sequence
  source: /note="Description of Artificial Sequence: Synthetic primer"
gaagtttaaaagagtgggaacatgggg

SEQ ID NO: 354 - DNA, 26 bp, Artificial Sequence
  source: /note="Description of Artificial Sequence: Synthetic primer"
ctacgtaagcaaaaatgatcacgcac

SEQ ID NO: 355 - DNA, 25 bp, Artificial Sequence
  source: /note="Description of Artificial Sequence: Synthetic primer"
aacctgatggccctcattagtcctt

SEQ ID NO: 356 - DNA, 28 bp, Artificial Sequence
  source: /note="Description of Artificial Sequence: Synthetic primer"
caccagatttctaggaatagcatgtgag

SEQ ID NO: 357 - DNA, 25 bp, Artificial Sequence
  source: /note="Description of Artificial Sequence: Synthetic primer"
aagagcatagtgaggggttagacct

SEQ ID NO: 358 - DNA, 29 bp, Artificial Sequence
  source: /note="Description of Artificial Sequence: Synthetic primer"
ctttatatttagtgtagagatcagtctcc

SEQ ID NO: 359 - DNA, 27 bp, Artificial Sequence
  source: /note="Description of Artificial Sequence: Synthetic primer"
tgagtcctttacctaatcttggttgtc

SEQ ID NO: 360 - DNA, 27 bp, Artificial Sequence
  source: /note="Description of Artificial Sequence: Synthetic primer"
aatccaaagcaactctcttttcaccac

SEQ ID NO: 361 - DNA, 26 bp, Artificial Sequence
  source: /note="Description of Artificial Sequence: Synthetic primer"
tttactggaaccctgattttgttgga

SEQ ID NO: 362 - DNA, 26 bp, Artificial Sequence
  source: /note="Description of Artificial Sequence: Synthetic primer"
tgccactgatatatcagtacctgagt

SEQ ID NO: 363 - DNA, 27 bp, Artificial Sequence
  source: /note="Description of Artificial Sequence: Synthetic primer"
acaatctcaatcccccttaatgttttc

SEQ ID NO: 364 - DNA, 25 bp, Artificial Sequence
  source: /note="Description of Artificial Sequence: Synthetic primer"
gtgggcagagagagtaagagaacct

SEQ ID NO: 365 - DNA, 28 bp, Artificial Sequence
  source: /note="Description of Artificial Sequence: Synthetic primer"
caaaccagattctggcagaatagttagc

SEQ ID NO: 366 - DNA, 25 bp, Artificial Sequence
  source: /note="Description of Artificial Sequence: Synthetic primer"
cttctctcccatcctccttctccac

SEQ ID NO: 367 - DNA, 27 bp, Artificial Sequence
  source: /note="Description of Artificial Sequence: Synthetic primer"
agatcaagggatctgtgggacaataac

SEQ ID NO: 368 - DNA, 26 bp, Artificial Sequence
  source: /note="Description of Artificial Sequence: Synthetic primer"
ggggagtgatttcaagcatcctgatt

SEQ ID NO: 369 - DNA, 27 bp, Artificial Sequence
  source: /note="Description of Artificial Sequence: Synthetic primer"
catgagtttgaggtaagatgaaggaga

SEQ ID NO: 370 - DNA, 26 bp, Artificial Sequence
  source: /note="Description of Artificial Sequence: Synthetic primer"
tctctctcatcctagtgaatgccatc

SEQ ID NO: 371 - DNA, 26 bp, Artificial Sequence
  source: /note="Description of Artificial Sequence: Synthetic primer"
gggtgatgatctaccttgcaggtata

SEQ ID NO: 372 - DNA, 25 bp, Artificial Sequence
  source: /note="Description of Artificial Sequence: Synthetic primer"
ctcaaggccctgggtctgaaattac

SEQ ID NO: 373 - DNA, 28 bp, Artificial Sequence
  source: /note="Description of Artificial Sequence: Synthetic primer"
acatctccagttaataatttccactaac

SEQ ID NO: 374 - DNA, 27 bp, Artificial Sequence
  source: /note="Description of Artificial Sequence: Synthetic primer"
tggattgctcaacaaatagtgctaaaa

SEQ ID NO: 375 - DNA, 27 bp, Artificial Sequence
  source: /note="Description of Artificial Sequence: Synthetic primer"
catgcgacatccaggtagctaaaatac

SEQ ID NO: 376 - DNA, 28 bp, Artificial Sequence
  source: /note="Description of Artificial Sequence: Synthetic primer"
atggataaaaatggaactttcaagagaa

SEQ ID NO: 377 - DNA, 28 bp, Artificial Sequence
  source: /note="Description of Artificial Sequence: Synthetic primer"
gttttatgtaaagcttcgtcatatggct

SEQ ID NO: 378 - DNA, 28 bp, Artificial Sequence
  source: /note="Description of Artificial Sequence: Synthetic primer"
gttccaacttagtcataaagttccctgg

SEQ ID NO: 379 - DNA, 28 bp, Artificial Sequence
  source: /note="Description of Artificial Sequence: Synthetic primer"
gggtcttgatgttgtattgatgaggaag

SEQ ID NO: 380 - DNA, 28 bp, Artificial Sequence
  source: /note="Description of Artificial Sequence: Synthetic primer"
cctaacagaaagtcactgtttgtatctg

SEQ ID NO: 381 - DNA, 26 bp, Artificial Sequence
  source: /note="Description of Artificial Sequence: Synthetic primer"
tcactctggcttgtactctctctgtg

SEQ ID NO: 382 - DNA, 28 bp, Artificial Sequence
  source: /note="Description of Artificial Sequence: Synthetic primer"
ggctggtttcagtctggagactttattt

SEQ ID NO: 383 - DNA, 27 bp, Artificial Sequence
  source: /note="Description of Artificial Sequence: Synthetic primer"
cttcacctcgatgacgatgatgatgat

SEQ ID NO: 384 - DNA, 28 bp, Artificial Sequence
  source: /note="Description of Artificial Sequence: Synthetic primer"
gacaataacagcacaaaggatggaaaag

SEQ ID NO: 385 - DNA, 25 bp, Artificial Sequence
  source: /note="Description of Artificial Sequence: Synthetic primer"
gaaccagaccacacaatatcaccac

SEQ ID NO: 386 - DNA, 28 bp, Artificial Sequence
  source: /note="Description of Artificial Sequence: Synthetic primer"
tctacctctttgatgtccccttcgatag

SEQ ID NO: 387 - DNA, 28 bp, Artificial Sequence
  source: /note="Description of Artificial Sequence: Synthetic primer"
cagagtttctcatctacgaaagaggagt

SEQ ID NO: 388 - DNA, 28 bp, Artificial Sequence
  source: /note="Description of Artificial Sequence: Synthetic primer"
cccagctttgaaaagtatgcctagaact

SEQ ID NO: 389 - DNA, 28 bp, Artificial Sequence
  source: /note="Description of Artificial Sequence: Synthetic primer"
ctgcttcaagtgtatataaactcacagt

SEQ ID NO: 390 - DNA, 28 bp, Artificial Sequence
  source: /note="Description of Artificial Sequence: Synthetic primer"
ttgtttcatccactttggtgggtaaaag

SEQ ID NO: 391 - DNA, 27 bp, Artificial Sequence
  source: /note="Description of Artificial Sequence: Synthetic primer"
taattaagctctgtgtttagggttttt

SEQ ID NO: 392 - DNA, 28 bp, Artificial Sequence
  source: /note="Description of Artificial Sequence: Synthetic primer"
caattctttgttctttaggtcagtatat

SEQ ID NO: 393 - DNA, 25 bp, Artificial Sequence
  source: /note="Description of Artificial Sequence: Synthetic primer"
tactcttcctcagtcccttctctgc

SEQ ID NO: 394 - DNA, 25 bp, Artificial Sequence
  source: /note="Description of Artificial Sequence: Synthetic primer"
tgagacagagcatgatgatcatggc

SEQ ID NO: 395 - DNA, 26 bp, Artificial Sequence
  source: /note="Description of Artificial Sequence: Synthetic primer"
gcacaagtctaggaactactttgcac

SEQ ID NO: 396 - DNA, 25 bp, Artificial Sequence
  source: /note="Description of Artificial Sequence: Synthetic primer"
gaagtatttgaaccatacggagccc

SEQ ID NO: 397 - DNA, 26 bp, Artificial Sequence
  source: /note="Description of Artificial Sequence: Synthetic primer"
tgaggaacacatccaaactatgacac

SEQ ID NO: 398 - DNA, 25 bp, Artificial Sequence
  source: /note="Description of Artificial Sequence: Synthetic primer"
tttctcgccctcatcatctgcaatg

SEQ ID NO: 399 - DNA, 27 bp, Artificial Sequence
  source: /note="Description of Artificial Sequence: Synthetic primer"
tcagttgatttcatgtgatcctcacag

SEQ ID NO: 400 - DNA, 27 bp, Artificial Sequence
  source: /note="Description of Artificial Sequence: Synthetic primer"
gaataaagtgaggaaaacacggagttg

SEQ ID NO: 401 - DNA, 28 bp, Artificial Sequence
  source: /note="Description of Artificial Sequence: Synthetic primer"
attaccttctttctaatacaagcatatg

SEQ ID NO: 402 - DNA, 28 bp, Artificial Sequence
  source: /note="Description of Artificial Sequence: Synthetic primer"
acaggaacaaagaatttgttcttcatgg

SEQ ID NO: 403 - DNA, 51 bp, Artificial Sequence
  source: /note="Description of Artificial Sequence: Synthetic primer"
  modified_base (22)..(26): a, c, t, g, unknown or other
tacacgacgctcttccgatctnnnnncaaagaagtcaaaacagagggatca

SEQ ID NO: 404 - DNA, 47 bp, Artificial Sequence
  source: /note="Description of Artificial Sequence: Synthetic primer"
  modified_base (22)..(26): a, c, t, g, unknown or other
tacacgacgctcttccgatctnnnnncaaaggcagatcccaagctct

SEQ ID NO: 405 - DNA, 48 bp, Artificial Sequence
  source: /note="Description of Artificial Sequence: Synthetic primer"
  modified_base (22)..(26): a, c, t, g, unknown or other
tacacgacgctcttccgatctnnnnncaatagtgtgcaaggatgggtg

SEQ ID NO: 406 - DNA, 52 bp, Artificial Sequence
  source: /note="Description of Artificial Sequence: Synthetic primer"
  modified_base (22)..(26): a, c, t, g, unknown or other
tacacgacgctcttccgatctnnnnncaacctaagctgaaatgcagatattc

SEQ ID NO: 407 - DNA, 45 bp, Artificial Sequence
  source: /note="Description of Artificial Sequence: Synthetic primer"
  modified_base (21)..(25): a, c, t, g, unknown or other
cttggcacccgagaattccannnnnaggaggttgaggctgcaaaa

SEQ ID NO: 408 - DNA, 46 bp, Artificial Sequence
  source: /note="Description of Artificial Sequence: Synthetic primer"
  modified_base (22)..(26): a, c, t, g, unknown or other
tacacgacgctcttccgatctnnnnngcatggtgaggctgaagtag

SEQ ID NO: 409 - DNA, 51 bp, Artificial Sequence
  source: /note="Description of Artificial Sequence: Synthetic primer"
  modified_base (22)..(26): a, c, t, g, unknown or other
tacacgacgctcttccgatctnnnnngcarctagaatataagcaggcagga

SEQ ID NO: 410 - DNA, 52 bp, Artificial Sequence
  source: /note="Description of Artificial Sequence: Synthetic primer"
  modified_base (22)..(26): a, c, t, g, unknown or other
tacacgacgctcttccgatctnnnnngcagtctcatttcctggagatgaagg

SEQ ID NO: 411 - DNA, 45 bp, Artificial Sequence
  source: /note="Description of Artificial Sequence: Synthetic primer"
  modified_base (22)..(26): a, c, t, g, unknown or other
tacacgacgctcttccgatctnnnnnccctgggctctgtaaagaa

SEQ ID NO: 412 - DNA, 51 bp, Artificial Sequence
  source: /note="Description of Artificial Sequence: Synthetic primer"
  modified_base (21)..(25): a, c, t, g, unknown or other
cttggcacccgagaattccannnnnggaacacaattatccctgagtagcag

SEQ ID NO: 413 - DNA, 47 bp, Artificial Sequence
  source: /note="Description of Artificial Sequence: Synthetic primer"
  modified_base (21)..(25): a, c, t, g, unknown or other
cttggcacccgagaattccannnnnggacagcctccatawccacatg

SEQ ID NO: 414 - DNA, 45 bp, Artificial Sequence
  source: /note="Description of Artificial Sequence: Synthetic primer"
  modified_base (21)..(25): a, c, t, g, unknown or other
cttggcacccgagaattccannnnngcatccrtgactctctggac

SEQ ID NO: 415 - DNA, 51 bp, Artificial Sequence
  source: /note="Description of Artificial Sequence: Synthetic primer"
  modified_base (22)..(26): a, c, t, g, unknown or other
tacacgacgctcttccgatctnnnnntgaaactaaagtcaaatggggctac

SEQ ID NO: 416 - DNA, 59 bp, Artificial Sequence
  source: /note="Description of Artificial Sequence: Synthetic primer"
  modified_base (27)..(29): a, c, t, g, unknown or other
tacacgacgctcttccgatcttacgbnnndcgcacaaagaagtcaaaacagagggatca

SEQ ID NO: 417 - DNA, 55 bp, Artificial Sequence
  source: /note="Description of Artificial Sequence: Synthetic primer"
  modified_base (27)..(29): a, c, t, g, unknown or other
tacacgacgctcttccgatcttacgbnnndcgctcaaaggcagatcccaagctct

SEQ ID NO: 418 - DNA, 56 bp, Artificial Sequence
  source: /note="Description of Artificial Sequence: Synthetic primer"
  modified_base (27)..(29): a, c, t, g, unknown or other
tacacgacgctcttccgatcttacgbnnndcgctcaatagtgtgcaaggatgggtg

SEQ ID NO: 419 - DNA, 60 bp, Artificial Sequence
  source: /note="Description of Artificial Sequence: Synthetic primer"
  modified_base (27)..(29): a, c, t, g, unknown or other
tacacgacgctcttccgatcttacgbnnndcgctcaacctaagctgaaatgcagatattc

SEQ ID NO: 420 - DNA, 52 bp, Artificial Sequence
  source: /note="Description of Artificial Sequence: Synthetic primer"
  modified_base (24)..(27): a, c, t, g, unknown or other
cttggcacccgagaattccaacgnnnnhccggaggaggttgaggctgcaaaa

SEQ ID NO: 421 - DNA, 54 bp, Artificial Sequence
  source: /note="Description of Artificial Sequence: Synthetic primer"
  modified_base (27)..(29): a, c, t, g, unknown or other
tacacgacgctcttccgatcttacgbnnndcgctgcatggtgaggctgaagtag

SEQ ID NO: 422 - DNA, 59 bp, Artificial Sequence
  source: /note="Description of Artificial Sequence: Synthetic primer"
  modified_base (27)..(29): a, c, t, g, unknown or other
tacacgacgctcttccgatcttacgbnnndcgctgcarctagaatataagcaggcagga

SEQ ID NO: 423 - DNA, 60 bp, Artificial Sequence
  source: /note="Description of Artificial Sequence: Synthetic primer"
  modified_base (27)..(29): a, c, t, g, unknown or other
tacacgacgctcttccgatcttacgbnnndcgctgcagtctcatttcctggagatgaagg

SEQ ID NO: 424 - DNA, 53 bp, Artificial Sequence
  source: /note="Description of Artificial Sequence: Synthetic primer"
  modified_base (27)..(29): a, c, t, g, unknown or other
tacacgacgctcttccgatcttacgbnnndcgctccctgggctctgtaaagaa

SEQ ID NO: 425 - DNA, 58 bp, Artificial Sequence
  source: /note="Description of Artificial Sequence: Synthetic primer"
  modified_base (24)..(27): a, c, t, g, unknown or other
cttggcacccgagaattccaacgnnnnhccgcggaacacaattatccctgagtagcag

SEQ ID NO: 426 - DNA, 54 bp, Artificial Sequence
  source: /note="Description of Artificial Sequence: Synthetic primer"
  modified_base (24)..(27): a, c, t, g, unknown or other
cttggcacccgagaattccaacgnnnnhccgcggacagcctccatawccacatg

SEQ ID NO: 427 - DNA, 52 bp, Artificial Sequence
  source: /note="Description of Artificial Sequence: Synthetic primer"
  modified_base (24)..(27): a, c, t, g, unknown or other
cttggcacccgagaattccaacgnnnnhccgcgcatccrtgactctctggac

SEQ ID NO: 428 - DNA, 59 bp, Artificial Sequence
  source: /note="Description of Artificial Sequence: Synthetic primer"
  modified_base (27)..(29): a, c, t, g, unknown or other
tacacgacgctcttccgatcttacgbnnndcgcctgaaactaaagtcaaatggggctac

SEQ ID NO: 429 - DNA, 24 bp, Artificial Sequence
  source: /note="Description of Artificial Sequence: Synthetic primer"
aatagagatcgcgagacagaaagg

SEQ ID NO: 430 - DNA, 29 bp, Artificial Sequence
  source: /note="Description of Artificial Sequence: Synthetic primer"
  modified_base (1)..(5): a, c, t, g, unknown or other
nnnnntttatggtctcagtgcccctcaga

SEQ ID NO: 431 - DNA, 23 bp, Artificial Sequence
  source: /note="Description of Artificial Sequence: Synthetic primer"
tgtgtggcagaagttgaaaatta

SEQ ID NO: 432 - DNA, 29 bp, Artificial Sequence
  source: /note="Description of Artificial Sequence: Synthetic primer"
  modified_base (1)..(5): a, c, t, g, unknown or other
nnnnntttatggtctcagtgcccctcaga

SEQ ID NO: 433 - DNA, 25 bp, Artificial Sequence
  source: /note="Description of Artificial Sequence: Synthetic primer"
ataaatcagaccaggatgaaagttc

SEQ ID NO: 434 - DNA, 29 bp, Artificial Sequence
  source: /note="Description of Artificial Sequence: Synthetic primer"
  modified_base (1)..(5): a, c, t, g, unknown or other
nnnnntttatggtctcagtgcccctcaga

SEQ ID NO: 435 - DNA, 28 bp, Artificial Sequence
  source: /note="Description of Artificial Sequence: Synthetic primer"
aataatcctcaaaaacaaagaaacatgg

SEQ ID NO: 436 - DNA, 29 bp, Artificial Sequence
  source: /note="Description of Artificial Sequence: Synthetic primer"
  modified_base (1)..(5): a, c, t, g, unknown or other
nnnnntttatggtctcagtgcccctcaga

SEQ ID NO: 437 - DNA, 20 bp, Artificial Sequence
  source: /note="Description of Artificial Sequence: Synthetic primer"
tctggcgaagtaacccaaac

SEQ ID NO: 438 - DNA, 29 bp, Artificial Sequence
  source: /note="Description of Artificial Sequence: Synthetic primer"
  modified_base (1)..(5): a, c, t, g, unknown or other
nnnnntttatggtctcagtgcccctcaga

SEQ ID NO: 439 - DNA, 25 bp, Artificial Sequence
  source: /note="Description of Artificial Sequence: Synthetic primer"
aaaacatgaagataacaaatcccaa

SEQ ID NO: 440 - DNA, 29 bp, Artificial Sequence
  source: /note="Description of Artificial Sequence: Synthetic primer"
  modified_base (1)..(5): a, c, t, g, unknown or other
nnnnntttatggtctcagtgcccctcaga

SEQ ID NO: 441 - DNA, 26 bp, Artificial Sequence
  source: /note="Description of Artificial Sequence: Synthetic primer"
  modified_base (22)..(26): a, c, t, g, unknown or other
tacacgacgctcttccgatctnnnnn

SEQ ID NO: 442 - DNA, 49 bp, Artificial Sequence
  source: /note="Description of Artificial Sequence: Synthetic primer"
  modified_base (21)..(25): a, c, t, g, unknown or other
cttggcacccgagaattccannnnntttatggtctcagtgcccctcaga

SEQ ID NO: 443 - DNA, 29 bp, Artificial Sequence
  source: /note="Description of Artificial Sequence: Synthetic primer"
  modified_base (25)..(29): a, c, t, g, unknown or other
tacacgacgctcttccgatctacgnnnnn

SEQ ID NO: 444 - DNA, 49 bp, Artificial Sequence; identical to SEQ ID NO: 442
  source: /note="Description of Artificial Sequence: Synthetic primer"
  modified_base (21)..(25): a, c, t, g, unknown or other

SEQ ID NO: 445 - DNA, 33 bp, Artificial Sequence
  source: /note="Description of Artificial Sequence: Synthetic primer"
  modified_base (25)..(29): a, c, t, g, unknown or other
tacacgacgctcttccgatctacgnnnnncgcg

SEQ ID NO: 446 - DNA, 52 bp, Artificial Sequence
  source: /note="Description of Artificial Sequence: Synthetic primer"
  modified_base (24)..(28): a, c, t, g, unknown or other
cttggcacccgagaattccaacgnnnnncgcgaaattgtggmcaggtgcggt

SEQ ID NO: 447 - DNA, 33 bp, Artificial Sequence
  source: /note="Description of Artificial Sequence: Synthetic primer"
  modified_base (25)..(28): a, c, t, g, unknown or other
tacacgacgctcttccgatctacgnnnndcgcg

SEQ ID NO: 448 - DNA, 52 bp, Artificial Sequence; identical to SEQ ID NO: 446
  source: /note="Description of Artificial Sequence: Synthetic primer"
  modified_base (24)..(28): a, c, t, g, unknown or other

SEQ ID NO: 449 - DNA, 51 bp, Artificial Sequence; identical to SEQ ID NO: 409
  source: /note="Description of Artificial Sequence: Synthetic primer"
  modified_base (22)..(26): a, c, t, g, unknown or other

SEQ ID NO: 450 - DNA, 49 bp, Artificial Sequence; identical to SEQ ID NO: 442
  source: /note="Description of Artificial Sequence: Synthetic primer"
  modified_base (21)..(25): a, c, t, g, unknown or other

SEQ ID NO: 451 - DNA, 31 bp, Artificial Sequence
  source: /note="Description of Artificial Sequence: Synthetic oligonucleotide"
actctttccctacacgacgctcttccgatct

SEQ ID NO: 452 - DNA, 67 bp, Artificial Sequence
  source: /note="Description of Artificial Sequence: Synthetic oligonucleotide"
  modified_base (21)..(25): a, c, t, g, unknown or other
cttggcacccgagaattccannnnntttatggtctcagtgcccctcagatcggaagagcgtcgtgta

SEQ ID NO: 453 - DNA, 77 bp, Artificial Sequence
  source: /note="Description of Artificial Sequence: Synthetic oligonucleotide"
  modified_base (53)..(57): a, c, t, g, unknown or other
actctttccctacacgacgctcttccgatctgaggggcactgagaccataaannnnntggaattctcgggtgccaag

SEQ ID NO: 454 - DNA, 30 bp, Artificial Sequence
  source: /note="Description of Artificial Sequence: Synthetic oligonucleotide"
actggagttccttggcacccgagaattcca

SEQ ID NO: 455 - DNA, 87 bp, Artificial Sequence
  source: /note="Description of Artificial Sequence: Synthetic oligonucleotide"
  modified_base (53)..(57): a, c, t, g, unknown or other
actctttccctacacgacgctcttccgatctgaggggcactgagaccataaannnnntggaattctcgggtgccaaggaactccagt

SEQ ID NO: 456 - DNA, 87 bp, Artificial Sequence
  source: /note="Description of Artificial Sequence: Synthetic oligonucleotide"
  modified_base (31)..(35): a, c, t, g, unknown or other
actggagttccttggcacccgagaattccannnnntttatggtctcagtgcccctcagatcggaagagcgtcgtgtagggaaagagt

SEQ ID NO: 457 - DNA, 51 bp, Artificial Sequence; identical to SEQ ID NO: 409
  source: /note="Description of Artificial Sequence: Synthetic primer"
  modified_base (22)..(26): a, c, t, g, unknown or other

SEQ ID NO: 458 - DNA, 44 bp, Artificial Sequence
  source: /note="Description of Artificial Sequence: Synthetic primer"
cttggcacccgagaattccatttatggtctcagtgcccctcaga

SEQ ID NO: 459 - DNA, 51 bp, Artificial Sequence
  source: /note="Description of Artificial Sequence: Synthetic primer"
tacacgacgctcttccgatcthbhhhgcarctagaatataagcaggcagga

SEQ ID NO: 460 - DNA, 44 bp, Artificial Sequence; identical to SEQ ID NO: 458
  source: /note="Description of Artificial Sequence: Synthetic primer"

SEQ ID NO: 461 - DNA, 58 bp, Artificial Sequence
  source: /note="Description of Artificial Sequence: Synthetic primer"
  modified_base (25)..(29): a, c, t, g, unknown or other
tacacgacgctcttccgatctacannnnnagcggcarctagaatataagcaggcagga

SEQ ID NO: 462 - DNA, 44 bp, Artificial Sequence; identical to SEQ ID NO: 458
  source: /note="Description of Artificial Sequence: Synthetic primer"

SEQ ID NO: 463 - DNA, 58 bp, Artificial Sequence
  source: /note="Description of Artificial Sequence: Synthetic primer"
  modified_base (26)..(28): a, c, t, g, unknown or other
tacacgacgctcttccgatctacahnnnbagcggcarctagaatataagcaggcagga

SEQ ID NO: 464 - DNA, 44 bp, Artificial Sequence; identical to SEQ ID NO: 458
  source: /note="Description of Artificial Sequence: Synthetic primer"

SEQ ID NO: 465 - DNA, 45 bp, Artificial Sequence; identical to SEQ ID NO: 411
  source: /note="Description of Artificial Sequence: Synthetic primer"
  modified_base (22)..(26): a, c, t, g, unknown or other

SEQ ID NO: 466 - DNA, 41 bp, Artificial Sequence
  source: /note="Description of Artificial Sequence: Synthetic primer"
cttggcacccgagaattccataaggaactgcccagggtcac

SEQ ID NO: 467 - DNA, 52 bp, Artificial Sequence
  source: /note="Description of Artificial Sequence: Synthetic primer"
  modified_base (26)..(28): a, c, t, g, unknown or other
tacacgacgctcttccgatctacgbnnndcgctccctgggctctgtaaagaa

SEQ ID NO: 468 - DNA, 41 bp, Artificial Sequence; identical to SEQ ID NO: 466
  source: /note="Description of Artificial Sequence: Synthetic primer"